European Patent Specification EP 3 700 564 B1, published September 17, 2025. Title: IMMUNOSTIMULATORY COMPOSITIONS. Applicant: BAYER ANIMAL HEALTH GMBH. The sequence listing filed with the application follows.

SEQUENCE LISTING (269 sequences)

SEQ ID NO: 1 - DNA, 36 bp, Artificial Sequence
  source: /note="Description of Artificial Sequence: Synthetic oligonucleotide"
  /note="5'-Cholesteryl modified"
tggggttttttttgcgtttttgcgtttttgcgtttt

SEQ ID NO: 2 - skipped

SEQ ID NO: 3 - DNA, 24 bp, Artificial Sequence
  source: /note="Description of Artificial Sequence: Synthetic oligonucleotide"
  misc_feature (1)..(24): /note="Phosphorothioate linkage between nucleotides"
tcgtcgttttgtcgttttgtcgtt

SEQ ID NO: 4 - DNA, 24 bp, Artificial Sequence
  source: /note="Description of Artificial Sequence: Synthetic oligonucleotide"
tcgtcgttttgtcgttttgtcgtt

SEQ ID NO: 5 - DNA, 25 bp, Artificial Sequence
  source: /note="Description of Artificial Sequence: Synthetic oligonucleotide"
tcgtcgttttgtcgttttgtcgttg

SEQ ID NO: 6 - DNA, 26 bp, Artificial Sequence
  source: /note="Description of Artificial Sequence: Synthetic oligonucleotide"
tcgtcgttttgtcgttttgtcgttgg

SEQ ID NO: 7 - DNA, 27 bp, Artificial Sequence
  source: /note="Description of Artificial Sequence: Synthetic oligonucleotide"
tcgtcgttttgtcgttttgtcgttggg

SEQ ID NO: 8 - DNA, 28 bp, Artificial Sequence
  source: /note="Description of Artificial Sequence: Synthetic oligonucleotide"
tcgtcgttttgtcgttttgtcgttgggg

SEQ ID NO: 9 - DNA, 29 bp, Artificial Sequence
  source: /note="Description of Artificial Sequence: Synthetic oligonucleotide"
tcgtcgttttgtcgttttgtcgttggggg

SEQ ID NO: 10 - DNA, 30 bp, Artificial Sequence
  source: /note="Description of Artificial Sequence: Synthetic oligonucleotide"
tcgtcgttttgtcgttttgtcgttgggggg

SEQ ID NO: 11 - DNA, 31 bp, Artificial Sequence
  source: /note="Description of Artificial Sequence: Synthetic oligonucleotide"
tcgtcgttttgtcgttttgtcgttggggggg

SEQ ID NO: 12 - DNA, 32 bp, Artificial Sequence
  source: /note="Description of Artificial Sequence: Synthetic oligonucleotide"
tcgtcgttttgtcgttttgtcgttgggggggg

SEQ ID NO: 13 - DNA, 24 bp, Artificial Sequence
  source: /note="Description of Artificial Sequence: Synthetic oligonucleotide"
tcgtcgttttgtcgttttgtcgtt

SEQ ID NO: 14 - DNA, 25 bp, Artificial Sequence
  source: /note="Description of Artificial Sequence: Synthetic oligonucleotide"
gtcgtcgttttgtcgttttgtcgtt

SEQ ID NO: 15 - DNA, 26 bp, Artificial Sequence
  source: /note="Description of Artificial Sequence: Synthetic oligonucleotide"
ggtcgtcgttttgtcgttttgtcgtt

SEQ ID NO: 16 - DNA, 27 bp, Artificial Sequence
  source: /note="Description of Artificial Sequence: Synthetic oligonucleotide"
gggtcgtcgttttgtcgttttgtcgtt

SEQ ID NO: 17 - DNA, 28 bp, Artificial Sequence
  source: /note="Description of Artificial Sequence: Synthetic oligonucleotide"
ggggtcgtcgttttgtcgttttgtcgtt

SEQ ID NO: 18 - DNA, 29 bp, Artificial Sequence
  source: /note="Description of Artificial Sequence: Synthetic oligonucleotide"
gggggtcgtcgttttgtcgttttgtcgtt

SEQ ID NO: 19 - DNA, 30 bp, Artificial Sequence
  source: /note="Description of Artificial Sequence: Synthetic oligonucleotide"
ggggggtcgtcgttttgtcgttttgtcgtt

SEQ ID NO: 20 - DNA, 31 bp, Artificial Sequence
  source: /note="Description of Artificial Sequence: Synthetic oligonucleotide"
gggggggtcgtcgttttgtcgttttgtcgtt

SEQ ID NO: 21 - DNA, 32 bp, Artificial Sequence
  source: /note="Description of Artificial Sequence: Synthetic oligonucleotide"
ggggggggtcgtcgttttgtcgttttgtcgtt

SEQ ID NO: 22 - DNA, 30 bp, Artificial Sequence
  source: /note="Description of Artificial Sequence: Synthetic oligonucleotide"
aaaaaatcgtcgttttgtcgttttgtcgtt

SEQ ID NO: 23 - DNA, 30 bp, Artificial Sequence
  source: /note="Description of Artificial Sequence: Synthetic oligonucleotide"
cccccctcgtcgttttgtcgttttgtcgtt

SEQ ID NO: 24 - DNA, 30 bp, Artificial Sequence
  source: /note="Description of Artificial Sequence: Synthetic oligonucleotide"
tttttttcgtcgttttgtcgttttgtcgtt

SEQ ID NO: 25 - DNA, 30 bp, Artificial Sequence; identical to SEQ ID NO: 19
  source: /note="Description of Artificial Sequence: Synthetic oligonucleotide"
  modified_base (8)..(8): 5-methyl-cytidine
  modified_base (11)..(11): 5-methyl-cytidine
  modified_base (19)..(19): 5-methyl-cytidine
  modified_base (27)..(27): 5-methyl-cytidine

SEQ ID NO: 26 - DNA, 30 bp, Artificial Sequence
  source: /note="Description of Artificial Sequence: Synthetic oligonucleotide"
cccccctgctgcttttgtgcttttgtgctt

SEQ ID NO: 27 - DNA, 30 bp, Artificial Sequence
  source: /note="Description of Artificial Sequence: Synthetic oligonucleotide"
tttttttcatcattttgtcattttgtcatt

SEQ ID NO: 28 - DNA, 30 bp, Artificial Sequence
  source: /note="Description of Artificial Sequence: Synthetic oligonucleotide"
  misc_feature (1)..(30): /note="Phosphorothioate linkage between nucleotides"
tgggggtcgtcgttttgtcgttttgtcgtt

SEQ ID NO: 29 - DNA, 29 bp, Artificial Sequence
  source: /note="Description of Artificial Sequence: Synthetic oligonucleotide"
  misc_feature (1)..(29): /note="Phosphorothioate linkage between nucleotides"
tcgtcgttttgtcgttttgtcgttggggg

SEQ ID NO: 30 - DNA, 30 bp, Artificial Sequence
  source: /note="Description of Artificial Sequence: Synthetic oligonucleotide"
agggggtcgtcgttttgtcgttttgtcgtt

SEQ ID NO: 31 - DNA, 30 bp, Artificial Sequence
  source: /note="Description of Artificial Sequence: Synthetic oligonucleotide"
gaggggtcgtcgttttgtcgttttgtcgtt

SEQ ID NO: 32 - DNA, 30 bp, Artificial Sequence
  source: /note="Description of Artificial Sequence: Synthetic oligonucleotide"
ggagggtcgtcgttttgtcgttttgtcgtt

SEQ ID NO: 33 - DNA, 30 bp, Artificial Sequence
  source: /note="Description of Artificial Sequence: Synthetic oligonucleotide"
gggaggtcgtcgttttgtcgttttgtcgtt

SEQ ID NO: 34 - DNA, 30 bp, Artificial Sequence
  source: /note="Description of Artificial Sequence: Synthetic oligonucleotide"
ggggagtcgtcgttttgtcgttttgtcgtt

SEQ ID NO: 35 - DNA, 30 bp, Artificial Sequence
  source: /note="Description of Artificial Sequence: Synthetic oligonucleotide"
gggggatcgtcgttttgtcgttttgtcgtt

SEQ ID NO: 36 - DNA, 30 bp, Artificial Sequence
  source: /note="Description of Artificial Sequence: Synthetic oligonucleotide"
aaggggtcgtcgttttgtcgttttgtcgtt

SEQ ID NO: 37 - DNA, 30 bp, Artificial Sequence
  source: /note="Description of Artificial Sequence: Synthetic oligonucleotide"
gaagggtcgtcgttttgtcgttttgtcgtt

SEQ ID NO: 38 - DNA, 30 bp, Artificial Sequence
  source: /note="Description of Artificial Sequence: Synthetic oligonucleotide"
ggaaggtcgtcgttttgtcgttttgtcgtt

SEQ ID NO: 39 - DNA, 30 bp, Artificial Sequence
  source: /note="Description of Artificial Sequence: Synthetic oligonucleotide"
gggaagtcgtcgttttgtcgttttgtcgtt

SEQ ID NO: 40 - DNA, 30 bp, Artificial Sequence
  source: /note="Description of Artificial Sequence: Synthetic oligonucleotide"
ggggaatcgtcgttttgtcgttttgtcgtt

SEQ ID NO: 41 - DNA, 30 bp, Artificial Sequence
  source: /note="Description of Artificial Sequence: Synthetic oligonucleotide"
cgggggtcgtcgttttgtcgttttgtcgtt

SEQ ID NO: 42 - DNA, 30 bp, Artificial Sequence
  source: /note="Description of Artificial Sequence: Synthetic oligonucleotide"
gcggggtcgtcgttttgtcgttttgtcgtt

SEQ ID NO: 43 - DNA, 30 bp, Artificial Sequence
  source: /note="Description of Artificial Sequence: Synthetic oligonucleotide"
ggcgggtcgtcgttttgtcgttttgtcgtt

SEQ ID NO: 44 - DNA, 30 bp, Artificial Sequence
  source: /note="Description of Artificial Sequence: Synthetic oligonucleotide"
gggcggtcgtcgttttgtcgttttgtcgtt

SEQ ID NO: 45 - DNA, 30 bp, Artificial Sequence
  source: /note="Description of Artificial Sequence: Synthetic oligonucleotide"
ggggcgtcgtcgttttgtcgttttgtcgtt

SEQ ID NO: 46 - DNA, 30 bp, Artificial Sequence
  source: /note="Description of Artificial Sequence: Synthetic oligonucleotide"
gggggctcgtcgttttgtcgttttgtcgtt

SEQ ID NO: 47 - DNA, 30 bp, Artificial Sequence
  source: /note="Description of Artificial Sequence: Synthetic oligonucleotide"
ccggggtcgtcgttttgtcgttttgtcgtt

SEQ ID NO: 48 - DNA, 30 bp, Artificial Sequence
  source: /note="Description of Artificial Sequence: Synthetic oligonucleotide"
gccgggtcgtcgttttgtcgttttgtcgtt

SEQ ID NO: 49 - DNA, 30 bp, Artificial Sequence
  source: /note="Description of Artificial Sequence: Synthetic oligonucleotide"
ggccggtcgtcgttttgtcgttttgtcgtt

SEQ ID NO: 50 - DNA, 30 bp, Artificial Sequence
  source: /note="Description of Artificial Sequence: Synthetic oligonucleotide"
gggccgtcgtcgttttgtcgttttgtcgtt

SEQ ID NO: 51 - DNA, 30 bp, Artificial Sequence
  source: /note="Description of Artificial Sequence: Synthetic oligonucleotide"
ggggcctcgtcgttttgtcgttttgtcgtt

SEQ ID NO: 52 - DNA, 30 bp, Artificial Sequence; identical to SEQ ID NO: 28
  source: /note="Description of Artificial Sequence: Synthetic oligonucleotide"

SEQ ID NO: 53 - DNA, 30 bp, Artificial Sequence
  source: /note="Description of Artificial Sequence: Synthetic oligonucleotide"
gtggggtcgtcgttttgtcgttttgtcgtt

SEQ ID NO: 54 - DNA, 30 bp, Artificial Sequence
  source: /note="Description of Artificial Sequence: Synthetic oligonucleotide"
ggtgggtcgtcgttttgtcgttttgtcgtt

SEQ ID NO: 55 - DNA, 30 bp, Artificial Sequence
  source: /note="Description of Artificial Sequence: Synthetic oligonucleotide"
gggtggtcgtcgttttgtcgttttgtcgtt

SEQ ID NO: 56 - DNA, 30 bp, Artificial Sequence
  source: /note="Description of Artificial Sequence: Synthetic oligonucleotide"
ggggtgtcgtcgttttgtcgttttgtcgtt

SEQ ID NO: 57 - DNA, 30 bp, Artificial Sequence
  source: /note="Description of Artificial Sequence: Synthetic oligonucleotide"
gggggttcgtcgttttgtcgttttgtcgtt

SEQ ID NO: 58 - DNA, 30 bp, Artificial Sequence
  source: /note="Description of Artificial Sequence: Synthetic oligonucleotide"
ttggggtcgtcgttttgtcgttttgtcgtt

SEQ ID NO: 59 - DNA, 30 bp, Artificial Sequence
  source: /note="Description of Artificial Sequence: Synthetic oligonucleotide"
gttgggtcgtcgttttgtcgttttgtcgtt

SEQ ID NO: 60 - DNA, 30 bp, Artificial Sequence
  source: /note="Description of Artificial Sequence: Synthetic oligonucleotide"
ggttggtcgtcgttttgtcgttttgtcgtt

SEQ ID NO: 61 - DNA, 30 bp, Artificial Sequence
  source: /note="Description of Artificial Sequence: Synthetic oligonucleotide"
gggttgtcgtcgttttgtcgttttgtcgtt

SEQ ID NO: 62 - DNA, 30 bp, Artificial Sequence
  source: /note="Description of Artificial Sequence: Synthetic oligonucleotide"
ggggtttcgtcgttttgtcgttttgtcgtt

SEQ ID NO: 63 - DNA, 28 bp, Artificial Sequence
  source: /note="Description of Artificial Sequence: Synthetic oligonucleotide"
agggtcgtcgttttgtcgttttgtcgtt

SEQ ID NO: 64 - DNA, 28 bp, Artificial Sequence
  source: /note="Description of Artificial Sequence: Synthetic oligonucleotide"
gaggtcgtcgttttgtcgttttgtcgtt

SEQ ID NO: 65 - DNA, 28 bp, Artificial Sequence
  source: /note="Description of Artificial Sequence: Synthetic oligonucleotide"
ggagtcgtcgttttgtcgttttgtcgtt

SEQ ID NO: 66 - DNA, 28 bp, Artificial Sequence
  source: /note="Description of Artificial Sequence: Synthetic oligonucleotide"
gggatcgtcgttttgtcgttttgtcgtt

SEQ ID NO: 67 - DNA, 28 bp, Artificial Sequence
  source: /note="Description of Artificial Sequence: Synthetic oligonucleotide"
cgggtcgtcgttttgtcgttttgtcgtt

SEQ ID NO: 68 - DNA, 28 bp, Artificial Sequence
  source: /note="Description of Artificial Sequence: Synthetic oligonucleotide"
gcggtcgtcgttttgtcgttttgtcgtt

SEQ ID NO: 69 - DNA, 28 bp, Artificial Sequence
  source: /note="Description of Artificial Sequence: Synthetic oligonucleotide"
ggcgtcgtcgttttgtcgttttgtcgtt

SEQ ID NO: 70 - DNA, 28 bp, Artificial Sequence
  source: /note="Description of Artificial Sequence: Synthetic oligonucleotide"
gggctcgtcgttttgtcgttttgtcgtt

SEQ ID NO: 71 - DNA, 28 bp, Artificial Sequence
  source: /note="Description of Artificial Sequence: Synthetic oligonucleotide"
tgggtcgtcgttttgtcgttttgtcgtt

SEQ ID NO: 72 - DNA, 28 bp, Artificial Sequence
  source: /note="Description of Artificial Sequence: Synthetic oligonucleotide"
gtggtcgtcgttttgtcgttttgtcgtt

SEQ ID NO: 73 - DNA, 28 bp, Artificial Sequence
  source: /note="Description of Artificial Sequence: Synthetic oligonucleotide"
ggtgtcgtcgttttgtcgttttgtcgtt

SEQ ID NO: 74 - DNA, 28 bp, Artificial Sequence
  source: /note="Description of Artificial Sequence: Synthetic oligonucleotide"
gggttcgtcgttttgtcgttttgtcgtt

SEQ ID NO: 75 - DNA, 20 bp, Artificial Sequence
  source: /note="Description of Artificial Sequence: Synthetic oligonucleotide"
tccatgacgttcctgatgct

SEQ ID NO: 76 - DNA, 25 bp, Artificial Sequence
  source: /note="Description of Artificial Sequence: Synthetic oligonucleotide"
tccatgacgttcctgatgctggggg

SEQ ID NO: 77 - DNA, 24 bp, Artificial Sequence
  source: /note="Description of Artificial Sequence: Synthetic oligonucleotide"
ggggtccatgacgttcctgatgct

SEQ ID NO: 78 - DNA, 26 bp, Artificial Sequence
  source: /note="Description of Artificial Sequence: Synthetic oligonucleotide"
ggggggtccatgacgttcctgatgct

SEQ ID NO: 79 - DNA, 20 bp, Artificial Sequence
  source: /note="Description of Artificial Sequence: Synthetic oligonucleotide"
tccatgacgttcctgacgtt

SEQ ID NO: 80 - DNA, 25 bp, Artificial Sequence
  source: /note="Description of Artificial Sequence: Synthetic oligonucleotide"
tccatgacgttcctgacgttggggg

SEQ ID NO: 81 - DNA, 24 bp, Artificial Sequence
  source: /note="Description of Artificial Sequence: Synthetic oligonucleotide"
ggggtccatgacgttcctgacgtt

SEQ ID NO: 82 - DNA, 26 bp, Artificial Sequence
  source: /note="Description of Artificial Sequence: Synthetic oligonucleotide"
ggggggtccatgacgttcctgacgtt

SEQ ID NO: 83 - DNA, 23 bp, Artificial Sequence
  source: /note="Description of Artificial Sequence: Synthetic oligonucleotide"
tcgacgttcgtcgttcgtcgttc

SEQ ID NO: 84 - DNA, 28 bp, Artificial Sequence
  source: /note="Description of Artificial Sequence: Synthetic oligonucleotide"
tcgacgttcgtcgttcgtcgttcggggg

SEQ ID NO: 85 - DNA, 27 bp, Artificial Sequence
  source: /note="Description of Artificial Sequence: Synthetic oligonucleotide"
ggggtcgacgttcgtcgttcgtcgttc

SEQ ID NO: 86 - DNA, 29 bp, Artificial Sequence
  source: /note="Description of Artificial Sequence: Synthetic oligonucleotide"
ggggggtcgacgttcgtcgttcgtcgttc

SEQ ID NO: 87 - DNA, 26 bp, Artificial Sequence
  source: /note="Description of Artificial Sequence: Synthetic oligonucleotide"
tcgcgacgttcgcccgacgttcggta

SEQ ID NO: 88 - DNA, 31 bp, Artificial Sequence
  source: /note="Description of Artificial Sequence: Synthetic oligonucleotide"
tcgcgacgttcgcccgacgttcggtaggggg

SEQ ID NO: 89 - DNA, 30 bp, Artificial Sequence
  source: /note="Description of Artificial Sequence: Synthetic oligonucleotide"
ggggtcgcgacgttcgcccgacgttcggta

SEQ ID NO: 90 - DNA, 32 bp, Artificial Sequence
  source: /note="Description of Artificial Sequence: Synthetic oligonucleotide"
ggggggtcgcgacgttcgcccgacgttcggta

SEQ ID NO: 91 - DNA, 22 bp, Artificial Sequence
  source: /note="Description of Artificial Sequence: Synthetic oligonucleotide"
tcgtcgttttcggcgcgcgccg

SEQ ID NO: 92 - DNA, 26 bp, Artificial Sequence
  source: /note="Description of Artificial Sequence: Synthetic oligonucleotide"
ggggtcgtcgttttcggcgcgcgccg

SEQ ID NO: 93 - DNA, 28 bp, Artificial Sequence
  source: /note="Description of Artificial Sequence: Synthetic oligonucleotide"
ggggggtcgtcgttttcggcgcgcgccg

SEQ ID NO: 94 - DNA, 25 bp, Artificial Sequence
  source: /note="Description of Artificial Sequence: Synthetic oligonucleotide"
tcgtcgtcgttcgaacgacgttgat

SEQ ID NO: 95 - DNA, 30 bp, Artificial Sequence
  source: /note="Description of Artificial Sequence: Synthetic oligonucleotide"
tcgtcgtcgttcgaacgacgttgatggggg

SEQ ID NO: 96 - DNA, 29 bp, Artificial Sequence
  source: /note="Description of Artificial Sequence: Synthetic oligonucleotide"
ggggtcgtcgtcgttcgaacgacgttgat

SEQ ID NO: 97 - DNA, 31 bp, Artificial Sequence
  source: /note="Description of Artificial Sequence: Synthetic oligonucleotide"
ggggggtcgtcgtcgttcgaacgacgttgat

SEQ ID NO: 98 - DNA, 22 bp, Artificial Sequence
  source: /note="Description of Artificial Sequence: Synthetic oligonucleotide"
tcgtcgttgtcgttttgtcgtt

SEQ ID NO: 99 - DNA, 27 bp, Artificial Sequence
  source: /note="Description of Artificial Sequence: Synthetic oligonucleotide"
tcgtcgttgtcgttttgtcgttggggg

SEQ ID NO: 100 - DNA, 28 bp, Artificial Sequence
  source: /note="Description of Artificial Sequence: Synthetic oligonucleotide"
ggggggtcgtcgttgtcgttttgtcgtt

SEQ ID NO: 101 - DNA, 19 bp, Artificial Sequence
  source: /note="Description of Artificial Sequence: Synthetic oligonucleotide"
gatctcgctcgctcgctat

SEQ ID NO: 102 - DNA, 25 bp, Artificial Sequence
  source: /note="Description of Artificial Sequence: Synthetic oligonucleotide"
gggggggatctcgctcgctcgctat

SEQ ID NO: 103 - DNA, 21 bp, Artificial Sequence
  source: /note="Description of Artificial Sequence: Synthetic oligonucleotide"
tcgtcgacgtcgttcgttctc

SEQ ID NO: 104 - DNA, 27 bp, Artificial Sequence
  source: /note="Description of Artificial Sequence: Synthetic oligonucleotide"
ggggggtcgtcgacgtcgttcgttctc

SEQ ID NO: 105 - DNA, 29 bp, Artificial Sequence
  source: /note="Description of Artificial Sequence: Synthetic oligonucleotide"
tccatgacgttcctgcagttcctgacgtt

SEQ ID NO: 106 - DNA, 35 bp, Artificial Sequence
  source: /note="Description of Artificial Sequence: Synthetic oligonucleotide"
ggggggtccatgacgttcctgcagttcctgacgtt

SEQ ID NO: 107 - DNA, 20 bp, Artificial Sequence
  source: /note="Description of Artificial Sequence: Synthetic oligonucleotide"
tccacgacgttttcgacgtt

SEQ ID NO: 108 - DNA, 26 bp, Artificial Sequence
  source: /note="Description of Artificial Sequence: Synthetic oligonucleotide"
ggggggtccacgacgttttcgacgtt

SEQ ID NO: 109 - DNA, 28 bp, Artificial Sequence
  source: /note="Description of Artificial Sequence: Synthetic oligonucleotide"
tttttcgtcgttttgtcgttttgtcgtt

SEQ ID NO: 110 - DNA, 30 bp, Artificial Sequence
  source: /note="Description of Artificial Sequence: Synthetic oligonucleotide"
ttagggtcgtcgttttgtcgttttgtcgtt

SEQ ID NO: 111 - DNA, 36 bp, Artificial Sequence
  source: /note="Description of Artificial Sequence: Synthetic oligonucleotide"
ttagggttagggtcgtcgttttgtcgttttgtcgtt

SEQ ID NO: 112 - DNA, 32 bp, Artificial Sequence
  source: /note="Description of Artificial Sequence: Synthetic oligonucleotide"
ttttggggtcgtcgttttgtcgttttgtcgtt

SEQ ID NO: 113 - DNA, 32 bp, Artificial Sequence
  source: /note="Description of Artificial Sequence: Synthetic oligonucleotide"
ggggtttttcgtcgttttgtcgttttgtcgtt

SEQ ID NO: 114 - DNA, 36 bp, Artificial Sequence
  source: /note="Description of Artificial Sequence: Synthetic oligonucleotide"
ggggttttggggtcgtcgttttgtcgttttgtcgtt

SEQ ID NO: 115 - DNA, 34 bp, Artificial Sequence
  source: /note="Description of Artificial Sequence: Synthetic oligonucleotide"
ttagggtttttcgtcgttttgtcgttttgtcgtt

SEQ ID NO: 116 - DNA, 40 bp, Artificial Sequence
  source: /note="Description of Artificial Sequence: Synthetic oligonucleotide"
ttagggttagggtttttcgtcgttttgtcgttttgtcgtt

SEQ ID NO: 117 - DNA, 44 bp, Artificial Sequence
  source: /note="Description of Artificial Sequence: Synthetic oligonucleotide"
tgtgggtgtgtgtgggtttttcgtcgttttgtcgttttgtcgtt

SEQ ID NO: 118 - DNA, 33 bp, Artificial Sequence
  source: /note="Description of Artificial Sequence: Synthetic oligonucleotide"
ggaggtttttcgtcgttttgtcgttttgtcgtt

SEQ ID NO: 119 - DNA, 35 bp, Artificial Sequence
  source: /note="Description of Artificial Sequence: Synthetic oligonucleotide"
tggaggctttttcgtcgttttgtcgttttgtcgtt

SEQ ID NO: 120 - DNA, 42 bp, Artificial Sequence
  source: /note="Description of Artificial Sequence: Synthetic oligonucleotide"
tggaggctggaggctttttcgtcgttttgtcgttttgtcgtt

SEQ ID NO: 121 - DNA, 46 bp, Artificial Sequence
  source: /note="Description of Artificial Sequence: Synthetic oligonucleotide"
gctgcgaggcgggtgggtgggatcgtcgttttgtcgttttgtcgtt

SEQ ID NO: 122 - DNA, 45 bp, Artificial Sequence
  source: /note="Description of Artificial Sequence: Synthetic oligonucleotide"
gctgcgggcgggtgggtgggatcgtcgttttgtcgttttgtcgtt

SEQ ID NO: 123 - DNA, 42 bp, Artificial Sequence
  source: /note="Description of Artificial Sequence: Synthetic oligonucleotide"
cgaggcgggtgggtgggatcgtcgttttgtcgttttgtcgtt

SEQ ID NO: 124 - DNA, 41 bp, Artificial Sequence
  source: /note="Description of Artificial Sequence: Synthetic oligonucleotide"
cgggcgggtgggtgggatcgtcgttttgtcgttttgtcgtt

SEQ ID NO: 125 - DNA, 42 bp, Artificial Sequence
  source: /note="Description of Artificial Sequence: Synthetic oligonucleotide"
gggcgtggtgggtggggttcgtcgttttgtcgttttgtcgtt

SEQ ID NO: 126 - DNA, 40 bp, Artificial Sequence
  source: /note="Description of Artificial Sequence: Synthetic oligonucleotide"
ggggtgggaggagggttcgtcgttttgtcgttttgtcgtt

SEQ ID NO: 127 - DNA, 44 bp, Artificial Sequence
  source: /note="Description of Artificial Sequence: Synthetic oligonucleotide"
ggggtcgggcgggccgggtgtcgtcgttttgtcgttttgtcgtt

SEQ ID NO: 128 - DNA, 48 bp, Artificial Sequence
  source: /note="Description of Artificial Sequence: Synthetic oligonucleotide"
ggtggtggggggggttggtagggttcgtcgttttgtcgttttgtcgtt

SEQ ID NO: 129 - DNA, 44 bp, Artificial Sequence
  source: /note="Description of Artificial Sequence: Synthetic oligonucleotide"
gggttagggttagggtagggtcgtcgttttgtcgttttgtcgtt

SEQ ID NO: 130 - DNA, 41 bp, Artificial Sequence
  source: /note="Description of Artificial Sequence: Synthetic oligonucleotide"
tgggggggtgggtgggttcgtcgttttgtcgttttgtcgtt

SEQ ID NO: 131 - DNA, 40 bp, Artificial Sequence
  source: /note="Description of Artificial Sequence: Synthetic oligonucleotide"
gggcgggcgggcgggctcgtcgttttgtcgttttgtcgtt

SEQ ID NO: 132 - DNA, 39 bp, Artificial Sequence
  source: /note="Description of Artificial Sequence: Synthetic oligonucleotide"
ggttggtgtggttggtcgtcgttttgtcgttttgtcgtt

SEQ ID NO: 133 - DNA, 42 bp, Artificial Sequence
  source: /note="Description of Artificial Sequence: Synthetic oligonucleotide"
ggtggatggcgcagtcggtcgtcgttttgtcgttttgtcgtt

SEQ ID NO: 134 - DNA, 44 bp, Artificial Sequence
  source: /note="Description of Artificial Sequence: Synthetic oligonucleotide"
tgggggtggacgggccgggttcgtcgttttgtcgttttgtcgtt

SEQ ID NO: 135 - DNA, 46 bp, Artificial Sequence
  source: /note="Description of Artificial Sequence: Synthetic oligonucleotide"
tgtgggggtggacgggccgggttcgtcgttttgtcgttttgtcgtt

SEQ ID NO: 136 - DNA, 45 bp, Artificial Sequence
  source: /note="Description of Artificial Sequence: Synthetic oligonucleotide"
gggttagggttagggttagggtcgtcgttttgtcgttttgtcgtt

SEQ ID NO: 137 - DNA, 47 bp, Artificial Sequence
  source: /note="Description of Artificial Sequence: Synthetic oligonucleotide"
gggcgcgggaggaagggggcgggtcgtcgttttgtcgttttgtcgtt

SEQ ID NO: 138 - DNA, 43 bp, Artificial Sequence
  source: /note="Description of Artificial Sequence: Synthetic oligonucleotide"
agggtggggagggtggggatcgtcgttttgtcgttttgtcgtt

SEQ ID NO: 139 - DNA, 46 bp, Artificial Sequence
  source: /note="Description of Artificial Sequence: Synthetic oligonucleotide"
agggagggcgctgggaggagggtcgtcgttttgtcgttttgtcgtt

SEQ ID NO: 140 - DNA, 44 bp, Artificial Sequence
  source: /note="Description of Artificial Sequence: Synthetic oligonucleotide"
ggggcgggccgggggcggggtcgtcgttttgtcgttttgtcgtt

SEQ ID NO: 141 - DNA, 34 bp, Artificial Sequence
  source: /note="Description of Artificial Sequence: Synthetic oligonucleotide"
ggggttggggtcgtcgttttgtcgttttgtcgtt

SEQ ID NO: 142 - DNA, 38 bp, Artificial Sequence
  source: /note="Description of Artificial Sequence: Synthetic oligonucleotide"
ggggttggggtttttcgtcgttttgtcgttttgtcgtt

SEQ ID NO: 143 - DNA, 30 bp, Artificial Sequence
  source: /note="Description of Artificial Sequence: Synthetic oligonucleotide"
tggggttcgtcgttttgtcgttttgtcgtt

SEQ ID NO: 144 - DNA, 14 bp, Artificial Sequence
  source: /note="Description of Artificial Sequence: Synthetic oligonucleotide"
tttttttacgattt

SEQ ID NO: 145 - DNA, 14 bp, Artificial Sequence
  source: /note="Description of Artificial Sequence: Synthetic oligonucleotide"
tttttttgcgattt

SEQ ID NO: 146 - DNA, 14 bp, Artificial Sequence
  source: /note="Description of Artificial Sequence: Synthetic oligonucleotide"
tttttttccgattt

SEQ ID NO: 147 - DNA, 14 bp, Artificial Sequence
  source: /note="Description of Artificial Sequence: Synthetic oligonucleotide"
ttttttttcgattt

SEQ ID NO: 148 - DNA, 14 bp, Artificial Sequence
  source: /note="Description of Artificial Sequence: Synthetic oligonucleotide"
tttttttacggttt

SEQ ID NO: 149 - DNA, 14 bp, Artificial Sequence
  source: /note="Description of Artificial Sequence: Synthetic oligonucleotide"
tttttttgcggttt

SEQ ID NO: 150 - DNA, 14 bp, Artificial Sequence
  source: /note="Description of Artificial Sequence: Synthetic oligonucleotide"
tttttttccggttt

SEQ ID NO: 151 - DNA, 14 bp, Artificial Sequence
  source: /note="Description of Artificial Sequence: Synthetic oligonucleotide"
ttttttttcggttt

SEQ ID NO: 152 - DNA, 14 bp, Artificial Sequence
  source: /note="Description of Artificial Sequence: Synthetic oligonucleotide"
tttttttacgcttt

SEQ ID NO: 153 - DNA, 14 bp, Artificial Sequence
  source: /note="Description of Artificial Sequence: Synthetic oligonucleotide"
tttttttgcgcttt

SEQ ID NO: 154 - DNA, 14 bp, Artificial Sequence
  source: /note="Description of Artificial Sequence: Synthetic oligonucleotide"
tttttttccgcttt

SEQ ID NO: 155 - DNA, 14 bp, Artificial Sequence
  source: /note="Description of Artificial Sequence: Synthetic oligonucleotide"
ttttttttcgcttt

SEQ ID NO: 156 - DNA, 14 bp, Artificial Sequence
  source: /note="Description of Artificial Sequence: Synthetic oligonucleotide"
tttttttacgtttt

SEQ ID NO: 157 - DNA, 14 bp, Artificial Sequence
  source: /note="Description of Artificial Sequence: Synthetic oligonucleotide"
tttttttgcgtttt

SEQ ID NO: 158 - DNA, 14 bp, Artificial Sequence
  source: /note="Description of Artificial Sequence: Synthetic oligonucleotide"
tttttttccgtttt

SEQ ID NO: 159 - DNA, 14 bp, Artificial Sequence
  source: /note="Description of Artificial Sequence: Synthetic oligonucleotide"
ttttttttcgtttt

SEQ ID NO: 160 - DNA, 20 bp, Artificial Sequence
  source: /note="Description of Artificial Sequence: Synthetic oligonucleotide"
ggggggtttttttacgattt

SEQ ID NO: 161 - DNA, 20 bp, Artificial Sequence
  source: /note="Description of Artificial Sequence: Synthetic oligonucleotide"
ggggggtttttttgcgattt

SEQ ID NO: 162 - DNA, 20 bp, Artificial Sequence
  source: /note="Description of Artificial Sequence: Synthetic oligonucleotide"
ggggggtttttttccgattt

SEQ ID NO: 163 - DNA, 20 bp, Artificial Sequence
  source: /note="Description of Artificial Sequence: Synthetic oligonucleotide"
ggggggttttttttcgattt

SEQ ID NO: 164 - DNA, 20 bp, Artificial Sequence
  source: /note="Description of Artificial Sequence: Synthetic oligonucleotide"
ggggggtttttttacggttt

SEQ ID NO: 165 - DNA, 20 bp, Artificial Sequence
  source: /note="Description of Artificial Sequence: Synthetic oligonucleotide"
ggggggtttttttgcggttt

SEQ ID NO: 166 - DNA, 20 bp, Artificial Sequence
  source: /note="Description of Artificial Sequence: Synthetic oligonucleotide"
ggggggtttttttccggttt

SEQ ID NO: 167 - DNA, 20 bp, Artificial Sequence
  source: /note="Description of Artificial Sequence: Synthetic oligonucleotide"
ggggggttttttttcggttt

SEQ ID NO: 168 - DNA, 20 bp, Artificial Sequence
  source: /note="Description of Artificial Sequence: Synthetic oligonucleotide"
ggggggtttttttacgcttt

SEQ ID NO: 169 - DNA, 20 bp, Artificial Sequence
  source: /note="Description of Artificial Sequence: Synthetic oligonucleotide"
ggggggtttttttgcgcttt

SEQ ID NO: 170 - DNA, 20 bp, Artificial Sequence
  source: /note="Description of Artificial Sequence: Synthetic oligonucleotide"
ggggggtttttttccgcttt

SEQ ID NO: 171 - DNA, 20 bp, Artificial Sequence
  source: /note="Description of Artificial Sequence: Synthetic oligonucleotide"
ggggggttttttttcgcttt

SEQ ID NO: 172 - DNA, 20 bp, Artificial Sequence
  source: /note="Description of Artificial Sequence: Synthetic oligonucleotide"
ggggggtttttttacgtttt

SEQ ID NO: 173 - DNA, 20 bp, Artificial Sequence
  source: /note="Description of Artificial Sequence: Synthetic oligonucleotide"
ggggggtttttttgcgtttt

SEQ ID NO: 174 - DNA, 20 bp, Artificial Sequence
  source: /note="Description of Artificial Sequence: Synthetic oligonucleotide"
ggggggtttttttccgtttt

SEQ ID NO: 175 - DNA, 20 bp, Artificial Sequence
  source: /note="Description of Artificial Sequence: Synthetic oligonucleotide"
ggggggttttttttcgtttt

SEQ ID NO: 176 - DNA, 28 bp, Artificial Sequence
  source: /note="Description of Artificial Sequence: Synthetic oligonucleotide"
ggggttggggtttttttttttacgattt

SEQ ID NO: 177 - DNA, 28 bp, Artificial Sequence
  source: /note="Description of Artificial Sequence: Synthetic oligonucleotide"
ggggttggggtttttttttttgcgattt

SEQ ID NO: 178 - DNA, 28 bp, Artificial Sequence
  source: /note="Description of Artificial Sequence: Synthetic oligonucleotide"
ggggttggggtttttttttttccgattt

SEQ ID NO: 179 - DNA, 28 bp, Artificial Sequence
  source: /note="Description of Artificial Sequence: Synthetic oligonucleotide"
ggggttggggttttttttttttcgattt

SEQ ID NO: 180 - DNA, 28 bp, Artificial Sequence
  source: /note="Description of Artificial Sequence: Synthetic oligonucleotide"
ggggttggggtttttttttttacggttt

SEQ ID NO: 181 - DNA, 28 bp, Artificial Sequence
  source: /note="Description of Artificial Sequence: Synthetic oligonucleotide"
ggggttggggtttttttttttgcggttt

SEQ ID NO: 182 - DNA, 28 bp, Artificial Sequence
  source: /note="Description of Artificial Sequence: Synthetic oligonucleotide"
ggggttggggtttttttttttccggttt

SEQ ID NO: 183 - DNA, 28 bp, Artificial Sequence
  source: /note="Description of Artificial Sequence: Synthetic oligonucleotide"
ggggttggggttttttttttttcggttt

SEQ ID NO: 184 - DNA, 28 bp, Artificial Sequence
  source: /note="Description of Artificial Sequence: Synthetic oligonucleotide"
ggggttggggtttttttttttacgcttt

SEQ ID NO: 185 - DNA, 28 bp, Artificial Sequence
  source: /note="Description of Artificial Sequence: Synthetic oligonucleotide"
ggggttggggtttttttttttgcgcttt

SEQ ID NO: 186 - DNA, 28 bp, Artificial Sequence
  source: /note="Description of Artificial Sequence: Synthetic oligonucleotide"
ggggttggggtttttttttttccgcttt

SEQ ID NO: 187 - DNA, 28 bp, Artificial Sequence
  source: /note="Description of Artificial Sequence: Synthetic oligonucleotide"
ggggttggggttttttttttttcgcttt

SEQ ID NO: 188 - DNA, 28 bp, Artificial Sequence
  source: /note="Description of Artificial Sequence: Synthetic oligonucleotide"
ggggttggggtttttttttttacgtttt

SEQ ID NO: 189 - DNA, 28 bp, Artificial Sequence
  source: /note="Description of Artificial Sequence: Synthetic oligonucleotide"
ggggttggggtttttttttttgcgtttt

SEQ ID NO: 190 - DNA, 28 bp, Artificial Sequence
  source: /note="Description of Artificial Sequence: Synthetic oligonucleotide"
ggggttggggtttttttttttccgtttt

SEQ ID NO: 191 - DNA, 28 bp, Artificial Sequence
  source: /note="Description of Artificial Sequence: Synthetic oligonucleotide"
ggggttggggttttttttttttcgtttt

SEQ ID NO: 192 - DNA, 28 bp, Artificial Sequence
  source: /note="Description of Artificial Sequence: Synthetic oligonucleotide"
ggggttggggtttttttttttggctttt

SEQ ID NO: 193 - DNA, 28 bp, Artificial Sequence
  source: /note="Description of Artificial Sequence: Synthetic oligonucleotide"
ggggttggggtttttttttttgtgtttt

SEQ ID NO: 194 - DNA, 28 bp, Artificial Sequence
  source: /note="Description of Artificial Sequence: Synthetic oligonucleotide"
ggggttggggtttttttttttgcatttt

SEQ ID NO: 195 - DNA, 27 bp, Artificial Sequence
  source: /note="Description of Artificial Sequence: Synthetic oligonucleotide"
ggggttggggttttttttttgcgtttt

SEQ ID NO: 196 - DNA, 26 bp, Artificial Sequence
  source: /note="Description of Artificial Sequence: Synthetic oligonucleotide"
ggggttggggtttttttttgcgtttt

SEQ ID NO: 197 - DNA, 25 bp, Artificial Sequence
  source: /note="Description of Artificial Sequence: Synthetic oligonucleotide"
ggggttggggttttttttgcgtttt

SEQ ID NO: 198 - DNA, 24 bp, Artificial Sequence
  source: /note="Description of Artificial Sequence: Synthetic oligonucleotide"
ggggttggggtttttttgcgtttt

SEQ ID NO: 199 - DNA, 23 bp, Artificial Sequence
  source: /note="Description of Artificial Sequence: Synthetic oligonucleotide"
ggggttggggttttttgcgtttt

SEQ ID NO: 200 - DNA, 22 bp, Artificial Sequence
  source: /note="Description of Artificial Sequence: Synthetic oligonucleotide"
ggggttggggtttttgcgtttt

SEQ ID NO: 201 - DNA, 27 bp, Artificial Sequence
  source: /note="Description of Artificial Sequence: Synthetic oligonucleotide"
ggggttggggtttttttttttgcgttt

SEQ ID NO: 202 - DNA, 26 bp, Artificial Sequence
  source: /note="Description of Artificial Sequence: Synthetic oligonucleotide"
ggggttggggtttttttttttgcgtt

SEQ ID NO: 203 - DNA, 25 bp, Artificial Sequence
  source: /note="Description of Artificial Sequence: Synthetic oligonucleotide"
ggggttggggtttttttttttgcgt

SEQ ID NO: 204 - DNA, 35 bp, Artificial Sequence
  source: /note="Description of Artificial Sequence: Synthetic oligonucleotide"
ggggttggggtttttttttttgcgttttgcgtttt

SEQ ID NO: 205 - DNA, 43 bp, Artificial Sequence
  source: /note="Description of Artificial Sequence: Synthetic oligonucleotide"
ggggttggggtttttttttttgcgttttgcgtttttgcgtttt

SEQ ID NO: 206 - DNA, 35 bp, Artificial Sequence
  source: /note="Description of Artificial Sequence: Synthetic oligonucleotide"
ggggttggggtttttttttttgcgatttgcgattt

SEQ ID NO: 207 - DNA, 42 bp, Artificial Sequence
  source: /note="Description of Artificial Sequence: Synthetic oligonucleotide"
ggggttggggtttttttttttgcgatttgcgatttgcgattt

SEQ ID NO: 208 - DNA, 35 bp, Artificial Sequence
  source: /note="Description of Artificial Sequence: Synthetic oligonucleotide"
ggggttggggtttttttttttacgctttacgcttt

SEQ ID NO: 209 - DNA, 42 bp, Artificial Sequence
  source: /note="Description of Artificial Sequence: Synthetic oligonucleotide"
ggggttggggtttttttttttacgctttacgctttacgcttt

SEQ ID NO: 210 - DNA, 35 bp, Artificial Sequence
  source: /note="Description of Artificial Sequence: Synthetic oligonucleotide"
ggggttggggttttttttttttcgcttttcgcttt

SEQ ID NO: 211 - DNA, 42 bp, Artificial Sequence
  source: /note="Description of Artificial Sequence: Synthetic oligonucleotide"
ggggttggggttttttttttttcgcttttcgcttttcgcttt

SEQ ID NO: 212 - DNA, 35 bp, Artificial Sequence
  source: /note="Description of Artificial Sequence: Synthetic oligonucleotide"
ggggttggggtttttttttttccgctttccgcttt

SEQ ID NO: 213 - DNA, 42 bp, Artificial Sequence
  source: /note="Description of Artificial Sequence: Synthetic oligonucleotide"
ggggttggggtttttttttttccgctttccgctttccgcttt

SEQ ID NO: 214 - DNA, 35 bp, Artificial Sequence
  source: /note="Description of Artificial Sequence: Synthetic oligonucleotide"
ggggttggggtttttttttttgcggtttgcggttt

SEQ ID NO: 215 - DNA, 42 bp, Artificial Sequence
  source: /note="Description of Artificial Sequence: Synthetic oligonucleotide"
ggggttggggtttttttttttgcggtttgcggtttgcggttt

SEQ ID NO: 216 - DNA, 27 bp, Artificial Sequence
  source: /note="Description of Artificial Sequence: Synthetic oligonucleotide"
ggggttggggttttttttcgcgcgttt

SEQ ID NO: 217 - DNA, 29 bp, Artificial Sequence
  source: /note="Description of Artificial Sequence: Synthetic oligonucleotide"
ggggttggggttttttttcgtcgtcgttt

SEQ ID NO: 218 - DNA, 31 bp, Artificial Sequence
  source: /note="Description of Artificial Sequence: Synthetic oligonucleotide"
ggggttggggttttttttcgttcgttcgttt

SEQ ID NO: 219 - DNA, 33 bp, Artificial Sequence
  source: /note="Description of Artificial Sequence: Synthetic oligonucleotide"
ggggttggggttttttttcgtttcgtttcgttt

SEQ ID NO: 220 - DNA, 35 bp, Artificial Sequence
  source: /note="Description of Artificial Sequence: Synthetic oligonucleotide"
ggggttggggttttttttcgttttcgttttcgttt

SEQ ID NO: 221 - DNA, 29 bp, Artificial Sequence
  source: /note="Description of Artificial Sequence: Synthetic oligonucleotide"
  modified_base (21)..(21): Abasic site
  modified_base (24)..(24): Abasic site
ggggttggggttttttttcgncgncgttt

SEQ ID NO: 222 - DNA, 20 bp, Artificial Sequence
  source: /note="Description of Artificial Sequence: Synthetic oligonucleotide"
ggggttggggttttttttcg

SEQ ID NO: 223 - DNA, 20 bp, Artificial Sequence
  source: /note="Description of Artificial Sequence: Synthetic oligonucleotide"
ggggttggggttttttttcg

SEQ ID NO: 224 - DNA, 34 bp, Artificial Sequence
  source: /note="Description of Artificial Sequence: Synthetic oligonucleotide"
ggggttggggttggggtttttttttttgcgtttt

SEQ ID NO: 225 - DNA, 20 bp, Artificial Sequence
  source: /note="Description of Artificial Sequence: Synthetic oligonucleotide"
ggggttggggttttttttcg

SEQ ID NO: 226 - DNA, 20 bp, Artificial Sequence
  source: /note="Description of Artificial Sequence: Synthetic oligonucleotide"
ggggttggggttttttttcg

SEQ ID NO: 227 - DNA, 20 bp, Artificial Sequence
  source: /note="Description of Artificial Sequence: Synthetic oligonucleotide"
ggggttggggttttttttcg

SEQ ID NO: 228 - DNA, 20 bp, Artificial Sequence
  source: /note="Description of Artificial Sequence: Synthetic oligonucleotide"
ggggttggggttttttttcg

SEQ ID NO: 229 - DNA, 15 bp, Artificial Sequence
  source: /note="Description of Artificial Sequence: Synthetic oligonucleotide"
tggggttttttttcg

SEQ ID NO: 230 - DNA, 15 bp, Artificial Sequence
  source: /note="Description of Artificial Sequence: Synthetic oligonucleotide"
tggggttttttttcg

SEQ ID NO: 231 - DNA, 15 bp, Artificial Sequence
  source: /note="Description of Artificial Sequence: Synthetic oligonucleotide"
tggggttttttttcg

SEQ ID NO: 232 - DNA, 15 bp, Artificial Sequence
  source: /note="Description of Artificial Sequence: Synthetic oligonucleotide"
tggggttttttttcg

SEQ ID NO: 233 - DNA, 15 bp, Artificial Sequence
  source: /note="Description of Artificial Sequence: Synthetic oligonucleotide"
tggggttttttttcg

SEQ ID NO: 234 - DNA, 20 bp, Artificial Sequence
  source: /note="Description of Artificial Sequence: Synthetic oligonucleotide"
ggggttggggttttttttcg

SEQ ID NO: 235 - DNA, 20 bp, Artificial Sequence
  source: /note="Description of Artificial Sequence: Synthetic oligonucleotide"
ggggttggggttttttttcg

SEQ ID NO: 236 - DNA, 20 bp, Artificial Sequence
  source: /note="Description of Artificial Sequence: Synthetic oligonucleotide"
ggggttggggttttttttcg

SEQ ID NO: 237 - DNA, 20 bp, Artificial Sequence
  source: /note="Description of Artificial Sequence: Synthetic oligonucleotide"
ggggttggggttttttttcg

SEQ ID NO: 238 - DNA, 20 bp, Artificial Sequence
  source: /note="Description of Artificial Sequence: Synthetic oligonucleotide"
ggggttggggttttttttcg

SEQ ID NO: 239 - DNA, 29 bp, Artificial Sequence
  source: /note="Description of Artificial Sequence: Synthetic oligonucleotide"
  modified_base (21)..(21): Abasic site
  modified_base (24)..(24): Abasic site
ggggttggggttttttttcgncgncgttt

SEQ ID NO: 240 - DNA, 20 bp, Artificial Sequence
  source: /note="Description of Artificial Sequence: Synthetic oligonucleotide"
ggggttggggttttttttcg

SEQ ID NO: 241 - DNA, 22 bp, Artificial Sequence
  source: /note="Description of Artificial Sequence: Synthetic oligonucleotide"
ggggttggggttttttttacgc

SEQ ID NO: 242 - DNA, 22 bp, Artificial Sequence
  source: /note="Description of Artificial Sequence: Synthetic oligonucleotide"
ggggttggggttttttttccgc

SEQ ID NO: 243 - DNA, 22 bp, Artificial Sequence
  source: /note="Description of Artificial Sequence: Synthetic oligonucleotide"
ggggttggggttttttttacgc

SEQ ID NO: 244 - DNA, 22 bp, Artificial Sequence
  source: /note="Description of Artificial Sequence: Synthetic oligonucleotide"
ggggttggggttttttttccgc

SEQ ID NO: 245 - DNA, 17 bp, Artificial Sequence
  source: /note="Description of Artificial Sequence: Synthetic oligonucleotide"
tggggttttttttacgc

SEQ ID NO: 246 - DNA, 17 bp, Artificial Sequence
  source: /note="Description of Artificial Sequence: Synthetic oligonucleotide"
tggggttttttttccgc

SEQ ID NO: 247 - DNA, 24 bp, Artificial Sequence
  source: /note="Description of Artificial Sequence: Synthetic oligonucleotide"
tcgtcgttttgtcgttttgtcgtt

SEQ ID NO: 248 - DNA, 24 bp, Artificial Sequence
  source: /note="Description of Artificial Sequence: Synthetic oligonucleotide"
tcgtcgttttgtcgttttgtcgtt

SEQ ID NO: 249 - DNA, 28 bp, Artificial Sequence
  source: /note="Description of Artificial Sequence: Synthetic oligonucleotide"
ggggtcgtcgttttgtcgttttgtcgtt

SEQ ID NO: 250 - DNA, 28 bp, Artificial Sequence
  source: /note="Description of Artificial Sequence: Synthetic oligonucleotide"
ggggtcgtcgttttgtcgttttgtcgtt

SEQ ID NO: 251 - DNA, 34 bp, Artificial Sequence
  source: /note="Description of Artificial Sequence: Synthetic oligonucleotide"
  /note="May be 3'-Cholesteryl modified"
tggggttttttcgtcgttttgtcgttttgtcgtt

SEQ ID NO: 252 - DNA, 36 bp, Artificial Sequence; identical to SEQ ID NO: 1
  source: /note="Description of Artificial Sequence: Synthetic oligonucleotide"

SEQ ID NO: 253 - DNA, 41 bp, Artificial Sequence
  source: /note="Description of Artificial Sequence: Synthetic oligonucleotide"
  /note="May be 5'-Cholesteryl modified"
ggggttggggttttttttgcgtttttgcgtttttgcgtttt

SEQ ID NO: 254 - DNA, 30 bp, Artificial Sequence
  source: /note="Description of Artificial Sequence: Synthetic oligonucleotide"
  /note="May be 5'-Cholesteryl modified"
tttttttgcgtttttgcgtttttgcgtttt

SEQ ID NO: 255 - DNA, 41 bp, Artificial Sequence
  source: /note="Description of Artificial Sequence: Synthetic oligonucleotide"
  /note="May be 5'-Cholesteryl modified"
ggggttggggttttttttccgcttttccgcttttccgcttt

SEQ ID NO: 256 - DNA, 30 bp, Artificial Sequence
  source: /note="Description of Artificial Sequence: Synthetic oligonucleotide"
  /note="May be 5'-Cholesteryl modified"
tttttttccgcttttccgcttttccgcttt

SEQ ID NO: 257 - DNA, 10 bp, Artificial Sequence
  source: /note="Description of Artificial Sequence: Synthetic oligonucleotide"
ggggttgggg

SEQ ID NO: 258 - DNA, 14 bp, Artificial Sequence
  source: /note="Description of Artificial Sequence: Synthetic oligonucleotide"
ggggttggggtttt

SEQ ID NO: 259-260 - skipped (2 entries)

SEQ ID NO: 261 - DNA, 12 bp, Artificial Sequence
  source: /note="Description of Artificial Sequence: Synthetic oligonucleotide"
ttagggttaggg

SEQ ID NO: 262 - DNA, 12 bp, Artificial Sequence
  source: /note="Description of Artificial Sequence: Synthetic oligonucleotide"
ggggttttgggg

SEQ ID NO: 263 - DNA, 16 bp, Artificial Sequence
  source: /note="Description of Artificial Sequence: Synthetic oligonucleotide"
ttagggttagggtttt

SEQ ID NO: 264 - DNA, 14 bp, Artificial Sequence
  source: /note="Description of Artificial Sequence: Synthetic oligonucleotide"
tggaggctggaggc

SEQ ID NO: 265 - DNA, 4242 bp, Artificial Sequence
  source: /note="Description of Artificial Sequence: Synthetic polynucleotide"
tgaccgcccaacgacccccgcccattgacgtcaataatgacgtatgttcccatagtaacgccaatagggactttccattgacgtcaatgggtggagtatttacggtaaactgcccacttggcagtacatcaagtgtatcatatgccaagtccgccccctattgacgtcaatgacggtaaatggcccgcctggcattatgcccagtacatgaccttacgggactttcctacttggcagtacatctacgtattagtcatcgctattaccatggtgatgcggttttggcagtacatcaatgggcgtggatagcggtttgactcacggggatttccaagtctccaccccattgacgtcaatgggagtttgttttggcaccaaaatcaacgggactttccaaaatgtcgtaacaactccgccccattgacgcaaatgggcggtaggcgtgtacggtgggaggtctatataagcagagctcgtttagtgaaccgtcagatcgcctggagacgccatccacgctgttttgacctccatagaagacaccgggaccgatccagcctcccctcgaagccgatctgataacggtaccgataagctggcggccgattaagctacagaagttggtcgtgaggcactgggcaggtaagtatcaaggttacaagacaggtttaaggagaccaatagaaactgggcttgtcgagacagagaagactcttgcgtttctgataggcacctattggtcttactgacatccactttgcctttctctccacaggtgtccactcccaggttcaattacagctcttaagcagccgcaagcttgatatcgaattcctgcagcccgggggatccactagttctagagcggccgccaccgcggtggagctcgaattatcagatcgattaataactatgctcaaaaattgtgtacctttagctttttaatttgtaaaggggttaataaggaatatttgatgtatagtgccttgactagagatcataatcagccataccacatttgtagaggttttacttgctttaaaaaacctcccacacctccccctgaacctgaaacataaaatgaatgcaattgttgttgttaacttgtttattgcagcttataatggttacaaataaagcaatagcatcacaaatttcacaaataaagcatttttttcactgcattctagttgtggtttgtccaaactcatcaatgtatcttatcatgtctggatcatcagatctgccggtctccctatagtgagtcgtattaatttcgataagccaggttaacctgcattaatgaatcggccaacgcgcggggagaggcggtttgcgtattgggcgctcttccgcttcctcgctcactgactcgctgcgctcggtcgttcggctgcggcgagcggtatcagctcactcaaaggcggtaatacggttatccacagaatcaggggataacgcaggaaagaacatgtgagcaaaaggccagcaaaaggccaggaaccgtaaaaaggccgcgttgctggcgtttttccataggctccgcccccctgacgagcatcacaaaaatcgacgctcaagtcagaggtggcgaaacccgacaggactataaagataccaggcgtttccccctggaagctccctcgtgcgctctcctgttccgaccctgccgcttaccggatacctgtccgcctttctcccttcgggaagcgtggcgctttctcatagctcacgctgtaggtatctcagttcggtgtaggtcgttcgctccaagctgggctgtgtgcacgaaccccccgttcagcccgaccgctgcgccttatccggtaactatcgtcttgagtccaacccggtaagacacgacttatcgccactggcagcagccactggtaacaggattagcagagcgaggtatgtaggcggtgctacagagttcttgaagtggtggcctaactacggctacactagaagaacagtatttggtatctgcgctctgctgaagccagttaccttcggaaaaagagttggtagctcttgatccggcaaacaaaccaccgctggtagcggtggtttttttgtttgcaagcagcagattacgcgcagaaaaaaaggatctcaagaagatcctttgatcttttctacggggtctgacgctcagtggaacgaaaactcacgttaagggattttggtcatgggcgcgcctaggcttttgcaaagatcgatcaagagacaggatgaggatcgtttcgcagcttttcattctgactgcaacgggcaataagtctctgtgtggattaaaaaaagagtgtctgatagcagcttctgaactggttacctgccgtgagtaaattaaaattttattgacttaggtcactaaggcgccttgcgctgaggttgcgtcgtgatatcatcagggcagaccggttacatccccctaacaagctgtataaagagaaatactatctcattggcgttgcccgcacctgacagtgcgacgttgggctgcgtccgtcgaccaacggtaccgaggtaacagcccaatctatccatgatctcggccaggccgggtcggccgttatgcagcccggctcgggtatgaagccattaaggagccgacccagcgcgaccgggcggccggtcacgctgcctctgctgaagcctgcctgtcactccctgcgcggcgtacccgccgttctcatcgagtaggctccggatcgcgaccccggacgggccctgggcccaggagcggcctatgacaaatgccgggtagcgatccggcattcagcattgactgcgcacggatccagtccttgcaggagccttatgccgaccgtagcaaaaaatgagcccgagccgatcgcgagttgtgatccggtcccgccgattgccggtcgcgatgacggtcctgtgtaagcgttatcgttaccaattgtttaagaagtatatacgctacgaggtacttgataacttctgcgtagcatacatgaggttttgtataaaaatggcgggcgatatcaacgcagtgtcagaaatccgaaacagtctgcgggactctggggttcgaaatgaccgaccaagcgacgcccaacctgccatcacgagatttcgattccaccgccgccttctatgaaaggttgggcttcggaatcgttttccgggacgccggctggatgatcctccagcgcggggatctcatgctggagttcttcgcccaccctaggcgcgctcatgagcggatacatatttgaatgtatttagaaaaataaacaaataggggttccgcgcacatttccccgaaaagtgccacctaaattgtaagcgttaatattttgttaaaattcgcgttaaatttttgttaaatcagctcattttttaaccaataggccgaaatcggcaaaatcccttataaatcaaaagaatagaccgagatagggttgagtgttgttccagtttggaacaagagtccactattaaagaacgtggactccaacgtcaaagggcgaaaaaccgtctatcagggcgatggcccactacgtgaaccatcaccctaatcaagttttttggggtcgaggtgccgtaaagcactaaatcggaaccctaaagggagcccccgatttagagcttgacggggaaagccggcgaacgtggcgagaaaggaagggaagaaagcgaaaggagcgggcgctagggcgctggcaagtgtagcggtcacgctgcgcgtaaccaccacacccgccgcgcttaatgcgccgctacagggcgcgtcccattcgccattcaggctgcgcaactgttgggaagggcgatcggtgcgggcctcttcgctattacgccagctggcgaaagggggatgtgctgcaaggcgattaagttgggtaacgccagggttttcccagtcacgacgttgtaaaacgacggccagtgagcgcgcgtaatacgactcactatagggcgaattgggtaccgggccccccctcgagcaggatctatacattgaatcaatattggcaattagccatattagtcattggttatatagcataaatcaatattggctattggccattgcatacgttgtatctatatcataatatgtacatttatattggctcatgtccaatatgaccgccatgttgacattgattattgactagttattaatagtaatcaattacggggtcattagttcatagcccatatatggagttccgcgttacataacttacggtaaatggcccgcctggc

SEQ ID NO: 266 - DNA, 4242 bp, Artificial Sequence
  source: /note="Description of Artificial Sequence: Synthetic polynucleotide"
ctaaattgtaagcgttaatattttgttaaaattcgcgttaaatttttgttaaatcagctcattttttaaccaataggccgaaatcggcaaaatcccttataaatcaaaagaatagaccgagatagggttgagtgttgttccagtttggaacaagagtccactattaaagaacgtggactccaacgtcaaagggcgaaaaaccgtctatcagggcgatggcccactacgtgaaccatcaccctaatcaagttttttggggtcgaggtgccgtaaagcactaaatcggaaccctaaagggagcccccgatttagagcttgacggggaaagccggcgaacgtggcgagaaaggaagggaagaaagcgaaaggagcgggcgctagggcgctggcaagtgtagcggtcacgctgcgcgtaaccaccacacccgccgcgcttaatgcgccgctacagggcgcgtcccattcgccattcaggctgcgcaactgttgggaagggcgatcggtgcgggcctcttcgctattacgccagctggcgaaagggggatgtgctgcaaggcgattaagttgggtaacgccagggttttcccagtcacgacgttgtaaaacgacggccagtgagcgcgcgtaatacgactcactatagggcgaattgggtaccgggccccccctcgagcaggatctatacattgaatcaatattggcaattagccatattagtcattggttatatagcataaatcaatattggctattggccattgcatacgttgtatctatatcataatatgtacatttatattggctcatgtccaatatgaccgccatgttgacattgattattgactagttattaatagtaatcaattacggggtcattagttcatagcccatatatggagttccgcgttacataacttacggtaaatggcccgcctggctgaccgcccaacgacccccgcccattgacgtcaataatgacgtatgttcccatagtaacgccaatagggactttccattgacgtcaatgggtggagtatttacggtaaactgcccacttggcagtacatcaagtgtatcatatgccaagtccgccccctattgacgtcaatgacggtaaatggcccgcctggcattatgcccagtacatgaccttacgggactttcctacttggcagtacatctacgtattagtcatcgctattaccatggtgatgcggttttggcagtacatcaatgggcgtggatagcggtttgactcacggggatttccaagtctccaccccattgacgtcaatgggagtttgttttggcaccaaaatcaacgggactttccaaaatgtcgtaacaactccgccccattgacgcaaatgggcggtaggcgtgtacggtgggaggtctatataagcagagctcgtttagtgaaccgtcagatcgcctggagacgccatccacgctgttttgacctccatagaagacaccgggaccgatccagcctcccctcgaagccgatctgataacggtaccgataagctggcggccgattaagctacagaagttggtcgtgaggcactgggcaggtaagtatcaaggttacaagacaggtttaaggagaccaatagaaactgggcttgtcgagacagagaagactcttgcgtttctgataggcacctattggtcttactgacatccactttgcctttctctccacaggtgtccactcccaggttcaattacagctcttaagcagccgcaagcttgatatcgaattcctgcagcccgggggatccactagttctagagcggccgccaccgcggtggagctcgaattatcagatcgattaataactatgctcaaaaattgtgtacctttagctttttaatttgtaaaggggttaataaggaatatttgatgtatagtgccttgactagagatcataatcagccataccacatttgtagaggttttacttgctttaaaaaacctcccacacctccccctgaacctgaaacataaaatgaatgcaattgttgttgttaacttgtttattgcagcttataatggttacaaataaagcaatagcatcacaaatttcacaaataaagcatttttttcactgcattctagttgtggtttgtccaaactcatcaatgtatcttatcatgtctggatcatcagatctgccggtctccctatagtgagtcgtattaatttcgataagccaggttaacctgcattaatgaatcggccaacgcgcggggagaggcggtttgcgtattgggcgctcttccgcttcctcgctcactgactcgctgcgctcggtcgttcggctgcggcgagcggtatcagctcactcaaaggcggtaatacggttatccacagaatcaggggataacgcaggaaagaacatgtgagcaaaaggccagcaaaaggccaggaaccgtaaaaaggccgcgttgctggcgtttttccataggctccgcccccctgacgagcatcacaaaaatcgacgctcaagtcagaggtggcgaaacccgacaggactataaagataccaggcgtttccccctggaagctccctcgtgcgctctcctgttccgaccctgccgcttaccggatacctgtccgcctttctcccttcgggaagcgtggcgctttctcatagctcacgctgtaggtatctcagttcggtgtaggtcgttcgctccaagctgggctgtgtgcacgaaccccccgttcagcccgaccgctgcgccttatccggtaactatcgtcttgagtccaacccggtaagacacgacttatcgccactggcagcagccactggtaacaggattagcagagcgaggtatgtaggcggtgctacagagttcttgaagtggtggcctaactacggctacactagaagaacagtatttggtatctgcgctctgctgaagccagttaccttcggaaaaagagttggtagctcttgatccggcaaacaaaccaccgctggtagcggtggtttttttgtttgcaagcagcagattacgcgcagaaaaaaaggatctcaagaagatcctttgatcttttctacggggtctgacgctcagtggaacgaaaactcacgttaagggattttggtcatgagcgcgcctaggcttttgcaaagatcgatcaagagacaggatgaggatcgtttcgcatgattgaacaagatggattgcacgcaggttctccggccgcttgggtggagaggctattcggctatgactgggcacaacagacaatcggctgctctgatgccgccgtgttccggctgtcagcgcaggggcgcccggttctttttgtcaagaccgacctgtccggtgccctgaatgaactgcaagacgaggcagcgcggctatcgtggctggccacgacgggcgttccttgcgcagctgtgctcgacgttgtcactgaagcgggaagggactggctgctattgggcgaagtgccggggcaggatctcctgtcatctcaccttgctcctgccgagaaagtatccatcatggctgatgcaatgcggcggctgcatacgcttgatccggctacctgcccattcgaccaccaagcgaaacatcgcatcgagcgagcacgtactcggatggaagccggtcttgtcgatcaggatgatctggacgaagagcatcaggggctcgcgccagccgaactgttcgccaggctcaaggcgagcatgcccgacggcgaggatctcgtcgtgacccatggcgatgcctgcttgccgaatatcatggtggaaaatggccgcttttctggattcatcgactgtggccggctgggtgtggcggaccgctatcaggacatagcgttggctacccgtgatattgctgaagagcttggcggcgaatgggctgaccgcttcctcgtgctttacggtatcgccgctcccgattcgcagcgcatcgccttctatcgccttcttgacgagttcttctgagcgggactctggggttcgaaatgaccgaccaagcgacgcccaacctgccatcacgagatttcgattccaccgccgccttctatgaaaggttgggcttcggaatcgttttccgggacgccggctggatgatcctccagcgcggggatctcatgctggagttcttcgcccaccctaggcgcgctcatgagcggatacatatttgaatgtatttagaaaaataaacaaataggggttccgcgcacatttccccgaaaagtgccac

SEQ ID NO: 267 - DNA, 4242 bp, Artificial Sequence
  source: /note="Description of Artificial Sequence: Synthetic polynucleotide"
tgaccgcccaacgacccccgcccattgacgtcaataatgacgtatgttcccatagtaacgccaatagggactttccattgacgtcaatgggtggagtatttacggtaaactgcccacttggcagtacatcaagtgtatcatatgccaagtccgccccctattgacgtcaatgacggtaaatggcccgcctggcattatgcccagtacatgaccttacgggactttcctacttggcagtacatctacgtattagtcatcgctattaccatggtgatgcggttttggcagtacatcaatgggcgtggatagcggtttgactcacggggatttccaagtctccaccccattgacgtcaatgggagtttgttttggcaccaaaatcaacgggactttccaaaatgtcgtaacaactccgccccattgacgcaaatgggcggtaggcgtgtacggtgggaggtctatataagcagagctcgtttagtgaaccgtcagatcgcctggagacgccatccacgctgttttgacctccatagaagacaccgggaccgatccagcctcccctcgaagccgatctgataacggtaccgataagctggcggccgattaagctacagaagttggtcgtgaggcactgggcaggtaagtatcaaggttacaagacaggtttaaggagaccaatagaaactgggcttgtcgagacagagaagactcttgcgtttctgataggcacctattggtcttactgacatccactttgcctttctctccacaggtgtccactcccaggttcaattacagctcttaagcagccgcaagcttgatatcgaattcctgcagcccgggggatccactagttctagagcggccgccaccgcggtggagctcgaattatcagatcgattaataactatgctcaaaaattgtgtacctttagctttttaatttgtaaaggggttaataaggaatatttgatgtatagtgccttgactagagatcataatcagccataccacatttgtagaggttttacttgctttaaaaaacctcccacacctccccctgaacctgaaacataaaatgaatgcaattgttgttgttaacttgtttattgcagcttataatggttacaaataaagcaatagcatcacaaatttcacaaataaagcatttttttcactgcattctagttgtggtttgtccaaactcatcaatgtatcttatcatgtctggatcatcagatctgccggtctccctatagtgagtcgtattaatttcgataagccaggttaacctgcattaatgaatcggccaacgcgcggggagaggcggtttgcgtattgggcgctcttccgcttcctcgctcactgactcgctgcgctcggtcgttcggctgcggcgagcggtatcagctcactcaaaggcggtaatacggttatccacagaatcaggggataacgcaggaaagaacatgtgagcaaaaggccagcaaaaggccaggaaccgtaaaaaggccgcgttgctggcgtttttccataggctccgcccccctgacgagcatcacaaaaatcgacgctcaagtcagaggtggcgaaacccgacaggactataaagataccaggcgtttccccctggaagctccctcgtgcgctctcctgttccgaccctgccgcttaccggatacctgtccgcctttctcccttcgggaagcgtggcgctttctcatagctcacgctgtaggtatctcagttcggtgtaggtcgttcgctccaagctgggctgtgtgcacgaaccccccgttcagcccgaccgctgcgccttatccggtaactatcgtcttgagtccaacccggtaagacacgacttatcgccactggcagcagccactggtaacaggattagcagagcgaggtatgtaggcggtgctacagagttcttgaagtggtggcctaactacggctacactagaagaacagtatttggtatctgcgctctgctgaagccagttaccttcggaaaaagagttggtagctcttgatccggcaaacaaaccaccgctggtagcggtggtttttttgtttgcaagcagcagattacgcgcagaaaaaaaggatctcaagaagatcctttgatcttttctacggggtctgacgctcagtggaacgaaaactcacgttaagggattttggtcatgggcgcgcctaggcttttgcaaagatcgatcaagagacaggatgaggatcgtttcgcatgattgaacaagatggattgcacgcaggttctccggccgcttgggtggagaggctattcggctatgactgggcacaacagacaatcggctgctctgatgccgccgtgttccggctgtcagcgcaggggcgcccggttctttttgtcaagaccgacctgtccggtgccctgaatgaactgcaagacgaggcagcgcggctatcgtggctggccacgacgggcgttccttgcgcagctgtgctcgacgttgtcactgaagcgggaagggactggctgctattgggcgaagtgccggggcaggatctcctgtcatctcaccttgctcctgccgagaaagtatccatcatggctgatgcaatgcggcggctgcatacgcttgatccggctacctgcccattcgaccaccaagcgaaacatcgcatcgagcgagcacgtactcggatggaagccggtcttgtcgatcaggatgatctggacgaagagcatcaggggctcgcgccagccgaactgttcgccaggctcaaggcgagcatgcccgacggcgaggatctcgtcgtgacccatggcgatgcctgcttgccgaatatcatggtggaaaatggccgcttttctggattcatcgactgtggccggctgggtgtggcggaccgctatcaggacatagcgttggctacccgtgatattgctgaagagcttggcggcgaatgggctgaccgcttcctcgtgctttacggtatcgccgctcccgattcgcagcgcatcgccttctatcgccttcttgacgagttcttctgagcgggactctggggttcgaaatgaccgaccaagcgacgcccaacctgccatcacgagatttcgattccaccgccgccttctatgaaaggttgggcttcggaatcgttttccgggacgccggctggatgatcctccagcgcggggatctcatgctggagttcttcgcccaccctaggcgcgctcatgagcggatacatatttgaatgtatttagaaaaataaacaaataggggttccgcgcacatttccccgaaaagtgccacctaaattgtaagcgttaatattttgttaaaattcgcgttaaatttttgttaaatcagctcattttttaaccaataggccgaaatcggcaaaatcccttataaatcaaaagaatagaccgagatagggttgagtgttgttccagtttggaacaagagtccactattaaagaacgtggactccaacgtcaaagggcgaaaaaccgtctatcagggcgatggcccactacgtgaaccatcaccctaatcaagttttttggggtcgaggtgccgtaaagcactaaatcggaaccctaaagggagcccccgatttagagcttgacggggaaagccggcgaacgtggcgagaaaggaagggaagaaagcgaaaggagcgggcgctagggcgctggcaagtgtagcggtcacgctgcgcgtaaccaccacacccgccgcgcttaatgcgccgctacagggcgcgtcccattcgccattcaggctgcgcaactgttgggaagggcgatcggtgcgggcctcttcgctattacgccagctggcgaaagggggatgtgctgcaaggcgattaagttgggtaacgccagggttttcccagtcacgacgttgtaaaacgacggccagtgagcgcgcgtaatacgactcactatagggcgaattgggtaccgggccccccctcgagcaggatctatacattgaatcaatattggcaattagccatattagtcattggttatatagcataaatcaatattggctattggccattgcatacgttgtatctatatcataatatgtacatttatattggctcatgtccaatatgaccgccatgttgacattgattattgactagttattaatagtaatcaattacggggtcattagttcatagcccatatatggagttccgcgttacataacttacggtaaatggcccgcctggc

SEQ ID NO: 268 - DNA, 4242 bp, Artificial Sequence
  source: /note="Description of Artificial Sequence: Synthetic polynucleotide"
tgaccgcccaacgacccccgcccattgacgtcaataatgacgtatgttcccatagtaacgccaatagggactttccattgacgtcaatgggtggagtatttacggtaaactgcccacttggcagtacatcaagtgtatcatatgccaagtccgccccctattgacgtcaatgacggtaaatggcccgcctggcattatgcccagtacatgaccttacgggactttcctacttggcagtacatctacgtattagtcatcgctattaccatggtgatgcggttttggcagtacatcaatgggcgtggatagcggtttgactcacggggatttccaagtctccaccccattgacgtcaatgggagtttgttttggcaccaaaatcaacgggactttccaaaatgtcgtaacaactccgccccattgacgcaaatgggcggtaggcgtgtacggtgggaggtctatataagcagagctcgtttagtgaaccgtcagatcgcctggagacgccatccacgctgttttgacctccatagaagacaccgggaccgatccagcctcccctcgaagccgatctgataacggtaccgataagctggcggccgattaagctacagaagttggtcgtgaggcactgggcaggtaagtatcaaggttacaagacaggtttaaggagaccaatagaaactgggcttgtcgagacagagaagactcttgcgtttctgataggcacctattggtcttactgacatccactttgcctttctctccacaggtgtccactcccaggttcaattacagctcttaagcagccgccaaaacaaaattcctcaaaaatcatcatcgaatgaatggtgaaataatttccctgaataactgtagtgttttcagggcgcggcataataattaactatgctcaaaaattgtgtacctttagctttttaatttgtaaaggggttaataaggaatatttgatgtatagtgccttgactagagatcataatcagccataccacatttgtagaggttttacttgctttaaaaaacctcccacacctccccctgaacctgaaacataaaatgaatgcaattgttgttgttaacttgtttattgcagcttataatggttacaaataaagcaatagcatcacaaatttcacaaataaagcatttttttcactgcattctagttgtggtttgtccaaactcatcaatgtatcttatcatgtctggatcatcagatctgccggtctccctatagtgagtcgtattaatttcgataagccaggttaacctgcattaatgaatcggccaacgcgcggggagaggcggtttgcgtattgggcgctcttccgcttcctcgctcactgactcgctgcgctcggtcgttcggctgcggcgagcggtatcagctcactcaaaggcggtaatacggttatccacagaatcaggggataacgcaggaaagaacatgtgagcaaaaggccagcaaaaggccaggaaccgtaaaaaggccgcgttgctggcgtttttccataggctccgcccccctgacgagcatcacaaaaatcgacgctcaagtcagaggtggcgaaacccgacaggactataaagataccaggcgtttccccctggaagctccctcgtgcgctctcctgttccgaccctgccgcttaccggatacctgtccgcctttctcccttcgggaagcgtggcgctttctcatagctcacgctgtaggtatctcagttcggtgtaggtcgttcgctccaagctgggctgtgtgcacgaaccccccgttcagcccgaccgctgcgccttatccggtaactatcgtcttgagtccaacccggtaagacacgacttatcgccactggcagcagccactggtaacaggattagcagagcgaggtatgtaggcggtgctacagagttcttgaagtggtggcctaactacggctacactagaagaacagtatttggtatctgcgctctgctgaagccagttaccttcggaaaaagagttggtagctcttgatccggcaaacaaaccaccgctggtagcggtggtttttttgtttgcaagcagcagattacgcgcagaaaaaaaggatctcaagaagatcctttgatcttttctacggggtctgacgctcagtggaacgaaaactcacgttaagggattttggtcatgggcgcgcctaggcttttgcaaagatcgatcaagagacaggatgaggatcgtttcgcagcttttcattctgactgcaacgggcaataagtctctgtgtggattaaaaaaagagtgtctgatagcagcttctgaactggttacctgccgtgagtaaattaaaattttattgacttaggtcactaaggcgccttgcgctgaggttgcgtcgtgatatcatcagggcagaccggttacatccccctaacaagctgtataaagagaaatactatctcattggcgttgcccgcacctgacagtgcgacgttgggctgcgtccgtcgaccaacggtaccgaggtaacagcccaatctatccatgatctcggccaggccgggtcggccgttatgcagcccggctcgggtatgaagccattaaggagccgacccagcgcgaccgggcggccggtcacgctgcctctgctgaagcctgcctgtcactccctgcgcggcgtacccgccgttctcatcgagtaggctccggatcgcgaccccggacgggccctgggcccaggagcggcctatgacaaatgccgggtagcgatccggcattcagcattgactgcgcacggatccagtccttgcaggagccttatgccgaccgtagcaaaaaatgagcccgagccgatcgcgagttgtgatccggtcccgccgattgccggtcgcgatgacggtcctgtgtaagcgttatcgttaccaattgtttaagaagtatatacgctacgaggtacttgataacttctgcgtagcatacatgaggttttgtataaaaatggcgggcgatatcaacgcagtgtcagaaatccgaaacagtctgcgggactctggggttcgaaatgaccgaccaagcgacgcccaacctgccatcacgagatttcgattccaccgccgccttctatgaaaggttgggcttcggaatcgttttccgggacgccggctggatgatcctccagcgcggggatctcatgctggagttcttcgcccaccctaggcgcgctcatgagcggatacatatttgaatgtatttagaaaaataaacaaataggggttccgcgcacatttccccgaaaagtgccacctaaattgtaagcgttaatattttgttaaaattcgcgttaaatttttgttaaatcagctcattttttaaccaataggccgaaatcggcaaaatcccttataaatcaaaagaatagaccgagatagggttgagtgttgttccagtttggaacaagagtccactattaaagaacgtggactccaacgtcaaagggcgaaaaaccgtctatcagggcgatggcccactacgtgaaccatcaccctaatcaagttttttggggtcgaggtgccgtaaagcactaaatcggaaccctaaagggagcccccgatttagagcttgacggggaaagccggcgaacgtggcgagaaaggaagggaagaaagcgaaaggagcgggcgctagggcgctggcaagtgtagcggtcacgctgcgcgtaaccaccacacccgccgcgcttaatgcgccgctacagggcgcgtcccattcgccattcaggctgcgcaactgttgggaagggcgatcggtgcgggcctcttcgctattacgccagctggcgaaagggggatgtgctgcaaggcgattaagttgggtaacgccagggttttcccagtcacgacgttgtaaaacgacggccagtgagcgcgcgtaatacgactcactatagggcgaattgggtaccgggccccccctcgaggtcgacggtatcgataagcttgatatcgaattcctgcagcccgggggatccactagttctagagcggccgccaccgcggtggagctccagcttttgttccctttagtgagggttaattgcgcgcttggcgtaatcatggtcatagctgtttcctgtgtgaaattgttatccgctcacaattccacacaacatacgagccggaagcataaagtgtaaagcctggggtgcctaatgagtgagctaactcacattaattgcgttgcgc

SEQ ID NO: 269 - DNA, 16 bp, Artificial Sequence
  source: /note="Description of Artificial Sequence: Synthetic oligonucleotide"
tgtgggtgtgtgtggg